European Patent Application EP 4 563 705 A1, published June 4, 2025. Title: Biocatalytic stereocontrolled production of 1-(R)-cis-PMD. Applicant: Universität Stuttgart. Application EP. The sequence listing filed with the application follows.

SEQUENCE LISTING (11 sequences)

SEQ ID NO: 1 - protein, 631 aa, Alicyclobacillus acidocaldarius
MAEQLVEAPAYARTLDRAVEYLLSCQKDEGYWWGPLLSNVTMEAEYVLLCHILDRVDRDRMEKIRRYLLHEQREDGTWALYPGGPPDLDTTIEAYVALKYIGMSRDEEPMQKALRFIQSQGGIESSRVFTRMWLALVGEYPWEKVPMVPPEIMFLGKRMPLNIYEFGSWARATVVAISIVMSRQPVFPLPERARVPELYDTDVPPRRRGAKGGGGRIFDALDRALHGYQKLSVHPFRRAAEIRALDWLLERQAGDGSWGGIQPPWFYTLIALKILDMTQHPAFIKGWEGLELYGVDLDYGGWMFQASISPVWDTGLAVLALRAAGLPADHDRLVKAGEWLLDRQITVPGDWAVKRPNLKPGGFAFQFDNVYYPDVDDTAVVVWALNSLRLPDERRRRDVMTKGFRWIVGMQSSNGGWGAYDVDNTSDLPNHIPFCDFGEVTDPPSEDVTAHVLECFGSFGYDDAWKVIRRAVEYLKREQRPDGSWFGRWGVNYLYGTGAVVPALKAVGIDVREPFIQKALDWVEQHQNPDGGWGEDCRSYEDPAYAGKGASTPSQTAWALMALIAGGRAESDSVRRGVQYLVETQRPDGGWDEPYYTGTGFPGDFYLGYTMYRHVFPTLALGRYKQAIERR

SEQ ID NO: 2 - protein, 680 aa, Streptomyces coelicolor
MTATTDGSTGASLRPLAASASDTDITIPAAAAGVPEAAARATRRATDFLLAKQDAEGWWKGDLETNVTMDAEDLLLRQFLGIQDEETTRAAALFIRGEQREDGTWATFYGGPGELSTTIEAYVALRLAGDSPEAPHMARAAEWIRSRGGIASARVFTRIWLALFGWWKWDDLPELPPELIYFPTWVPLNIYDFGCWARQTIVPLTIVSAKRPVRPAPFPLDELHTDPARPNPPRPLAPVASWDGAFQRIDKALHAYRKVAPRRLRRAAMNSAARWIIERQENDGCWGGIQPPAVYSVIALYLLGYDLEHPVMRAGLESLDRFAVWREDGARMIEACQSPVWDTCLATIALADAGVPEDHPQLVKASDWMLGEQIVRPGDWSVKRPGLPPGGWAFEFHNDNYPDIDDTAEVVLALRRVRHHDPERVEKAIGRGVRWNLGMQSKNGAWGAFDVDNTSAFPNRLPFCDFGEVIDPPSADVTAHVVEMLAVEGLAHDPRTRRGIQWLLDAQETDGSWFGRWGVNYVYGTGSVIPALTAAGLPTSHPAIRRAVRWLESVQNEDGGWGEDLRSYRYVREWSGRGASTASQTGWALMALLAAGERDSKAVERGVAWLAATQREDGSWDEPYFTGTGFPWDFSINYNLYRQVFPLTALGRYVHGEPFAKKPRAADAPAEAAPAEVKGS

SEQ ID NO: 3 - protein, 725 aa, Zymomonas mobilis
MGIDRMNSLSRLLMKKIFGAEKTSYKPASDTIIGTDTLKRPNRRPEPTAKVDKTIFKTMGNSLNNTLVSACDWLIGQQKPDGHWVGAVESNASMEAEWCLALWFLGLEDHPLRPRLGNALLEMQREDGSWGVYFGAGNGDINATVEAYAALRSLGYSADNPVLKKAAAWIAEKGGLKNIRVFTRYWLALIGEWPWEKTPNLPPEIIWFPDNFVFSIYNFAQWARATMVPIAILSARRPSRPLRPQDRLDELFPEGRARFDYELPKKEGIDLWSQFFRTTDRGLHWVQSNLLKRNSLREAAIRHVLEWIIRHQDADGGWGGIQPPWVYGLMALHGEGYQLYHPVMAKALSALDDPGWRHDRGESSWIQATNSPVWDTMLALMALKDAKAEDRFTPEMDKAADWLLARQVKVKGDWSIKLPDVEPGGWAFEYANDRYPDTDDTAVALIALSSYRDKEEWQKKGVEDAITRGVNWLIAMQSECGGWGAFDKDNNRSILSKIPFCDFGESIDPPSVDVTAHVLEAFGTLGLSRDMPVIQKAIDYVRSEQEAEGAWFGRWGVNYIYGTGAVLPALAAIGEDMTQPYITKACDWLVAHQQEDGGWGESCSSYMEIDSIGKGPTTPSQTAWALMGLIAANRPEDYEAIAKGCHYLIDRQEQDGSWKEEEFTGTGFPGYGVGQTIKLDDPALSKRLLQGAELSRAFMLRYDFYRQFFPIMALSRAERLIDLNN

SEQ ID NO: 4 - protein, 658 aa, Zymomonas mobilis
MTVSTSSAFHHSPLSDDVEPIIQKATRALLEKQQQDGHWVFELEADATIPAEYILLKHYLGEPEDLEIEAKIGRYLRRIQGEHGGWSLFYGGDLDLSATVKAYFALKMIGDSPDAPHMLRARNEILARGGAMRANVFTRIQLALFGAMSWEHVPQMPVELMLMPEWFPVHINKMAYWARTVLVPLLVLQALKPVARNRRGILVDELFVPDVLPTLQESGDPIWRRFFSALDKVLHKVEPYWPKNMRAKAIHSCVHFVTERLNGEDGLGAIYPAIANSVMMYDALGYPENHPERAIARRAVEKLMVLDGTEDQGDKEVYCQPCLSPIWDTALVAHAMLEVGGDEAEKSAISALSWLKPQQILDVKGDWAWRRPDLRPGGWAFQYRNDYYPDVDDTAVVTMAMDRAAKLSDLHDDFEESKARAMEWTIGMQSDNGGWGAFDANNSYTYLNNIPFADHGALLDPPTVDVSARCVSMMAQAGISITDPKMKAAVDYLLKEQEEDGSWFGRWGVNYIYGTWSALCALNVAALPHDHLAVQKAVAWLKTIQNEDGGWGENCDSYALDYSGYEPMDSTASQTAWALLGLMAVGEANSEAVTKGINWLAQNQDEEGLWKEDYYSGGGFPRVFYLRYHGYSKYFPLWALARYRNLKKANQPIVHYGM

SEQ ID NO: 5 - protein, 642 aa, Thermosynechococcus elongatus
MPTSLATAIDPKQLQQAIRASQDFLFSQQYAEGYWWAELESNVTMTAEVILLHKIWGTEQRLPLAKAEQYLRNHQRDHGGWELFYGDGGDLSTSVEAYMGLRLLGVPETDPALVKARQFILARGGISKTRIFTKLHLALIGCYDWRGIPSLPPWIMLLPEGSPFTIYEMSSWARSSTVPLLIVMDRKPVYGMDPPITLDELYSEGRANVVWELPRQGDWRDVFIGLDRVFKLFETLNIHPLREQGLKAAEEWVLERQEASGDWGGIIPAMLNSLLALRALDYAVDDPIVQRGMAAVDRFAIETETEYRVQPCVSPVWDTALVMRAMVDSGVAPDHPALVKAGEWLLSKQILDYGDWHIKNKKGRPGGWAFEFENRFYPDVDDTAVVVMALHAVTLPNENLKRRAIERAVAWIASMQCRPGGWAAFDVDNDQDWLNGIPYGDLKAMIDPNTADVTARVLEMVGRCQLAFDRVALDRALAYLRNEQEPEGCWFGRWGVNYLYGTSGVLTALSLVAPRYDRWRIRRAAEWLMQCQNADGGWGETCWSYHDPSLKGKGDSTASQTAWAIIGLLAAGDATGDYATEAIERGIAYLLETQRPDGTWHEDYFTGTGFPCHFYLKYHYYQQHFPLTALGRYARWRNLLAT

SEQ ID NO: 6 - protein, 631 aa, Alicyclobacillus acidocaldarius
MAEQLVEAPAYARTLDRAVEYLLSCQKDEGYWWGPLLSNVTMEAEYVLLCHILDRVDRDRMEKIRRYLLHEQREDGTWALYPGGPPDLDTTIEAYVALKYIGMSRDEEPMQKALRFIQSQGGIESSRVFTRMWLALVGEYPWEKVPMVPPEIMFLGKRMPLNIYEFGSWARATVVAISIVMSRQPVFPLPERARVPELYDTDVPPRRRGAKGGGGRIFDALDRALHGYQKLSVHPFRRAAEIRALDWLLERQAGDGSWGGIQPPWFYTLIALKILDMTQHPAFIKGWEGLELYGVDLDYGGWMFQASISPVWDTGLAVLALRAAGLPADHDRLVKAGEWLLDRQITVPGDWAVKRPNLKPGGFAAQFDNVYYPDVDDTAVVVWALNSLRLPDERRRRDVMTKGFRWIVGMQSSNGGWGAWDVDNTSDLPNHIPFCDFGEVTDPPSEDVTAHVLECFGSFGYDDAWKVIRRAVEYLKREQRPDGSWFGRWGVNYLYGTGAVVPALKAVGIDVREPFIQKALDWVEQHQNPDGGWGEDCRSYEDPAYAGKGASTPSQTAWALMALIAGGRAESDSVRRGVQYLVETQRPDGGWDEPYYTGTFFPGDFYLGYTMYRHVFPTLALGRYKQAIERR

SEQ ID NO: 7 - protein, 631 aa, Alicyclobacillus acidocaldarius
MAEQLVEAPAYARTLDRAVEYLLSCQKDEGYWWGPLLSNVTMEAEYVLLCHILDRVDRDRMEKIRRYLLHEQREDGTWALYPGGPPDLDTTIEAYVALKYIGMSRDEEPMQKALRFIQSQGGIESSRVFTRMWLALVGEYPWEKVPMVPPEIMFLGKRMPLNIYEFGSWARATVVAISIVMSRQPVFPLPERARVPELYDTDVPPRRRGAKGGGGRIFDALDRALHGYQKLSVHPFRRAAEIRALDWLLERQAGDGSWGGIQPPWFYTLIALKILDMTQHPAFIKGWEGLELYGVDLDYGGWMFQASISPVWDTGLAVLALRAAGLPADHDRLVKAGEWLLDRQITVPGDWAVKRPNLKPGGFAAQFDNVYYPDVDDTAVVVWALNSLRLPDERRRRDVMTKGFRWIVGMQSSNGGWGAYDVDNTSDLPNHIPFCDFGEVTDPPSEDVTAHVLECFGSFGYDDAWKVIRRAVEYLKREQRPDGSWFGRWGVNYLYGTGAVVPALKAVGIDVREPFIQKALDWVEQHQNPDGGWGEDCRSYEDPAYAGKGASTPSQTAWALMALIAGGRAESDSVRRGVQYLVETQRPDGGWDEPYYTGTGFPGDFYGGYTMYRHVFPTLALGRYKQAIERR

SEQ ID NO: 8 - protein, 631 aa, Alicyclobacillus acidocaldarius
MAEQLVEAPAYARTLDRAVEYLLSCQKDEGYWWGPLLSNVTMEAEYVLLCHILDRVDRDRMEKIRRYLLHEQREDGTWALYPGGPPDLDTTIEAYVALKYIGMSRDEEPMQKALRFIQSQGGIESSRVFTRMWLALVGEYPWEKVPMVPPEIMFLGKRMPLNIYEFGSWARATVVAISIVMSRQPVFPLPERARVPELYDTDVPPRRRGAKGGGGRIFDALDRALHGYQKLSVHPFRRAAEIRALDWLLERQAGDGSWGGIQPPWFYTLIALKILDMTQHPAFIKGWEGLELYGVDLDYGGWMFQASISPVWDTGLAVLALRAAGLPADHDRLVKAGEWLLDRQITVPGDWAVKRPNLKPGGFAAQFDNVYYPDVDDTAVVVWALNSLRLPDERRRRDVMTKGFRWIVGMQSSNGGWGAYDVDNTSDLPNHIPFCDFGEVTDPPSEDVTAHVLECFGSFGYDDAWKVIRRAVEYLKREQRPDGSWFGRWGVNYLYGTGAVVPALKAVGIDVREPFIQKALDWVEQHQNPDGGWGEDCRSYEDPAYAGKGASTPSQTAWALMALIAGGRAESDSVRRGVQYLVETQRPDGGWDEPYYTGTFFPGDFYGGYTMYRHVFPTLALGRYKQAIERR

SEQ ID NO: 9 - protein, 631 aa, Alicyclobacillus acidocaldarius
MAEQLVEAPAYARTLDRAVEYLLSCQKDEGYWWGPLLSNVTMEAEYVLLCHILDRVDRDRMEKIRRYLLHEQREDGTWALYPGGPPDLDTTIEAYVALKYIGMSRDEEPMQKALRFIQSQGGIESSRVFTRMWLALVGEYPWEKVPMVPPEIMFLGKRMPLNIYEFGSWARATVVAISIVMSRQPVFPLPERARVPELYDTDVPPRRRGAKGGGGRIFDALDRALHGYQKLSVHPFRRAAEIRALDWLLERQAGDGSWGGIQPPWFYTLIALKILDMTQHPAFIKGWEGLELYGVDLDYGGWMFQASISPVWDTGLAVLALRAAGLPADHDRLVKAGEWLLDRQITVPGDWAVKRPNLKPGGFAAQFDNVYYPDVDDTAVVVWALNSLRLPDERRRRDVMTKGFRWIVGMQSSNGGWGAYDVDNTSDLPNHIPFCDFGEVTDPPSEDVTAHVLECFGSFGYDDAWKVIRRAVEYLKREQRPDGSWFGRWGVNYLYGTGAVVPALKAVGIDVREPFIQKALDWVEQHQNPDGGWGEDCRSYEDPAYAGKGASTPSQTAWALMALIAGGRAESDSVRRGVQYLVETQRPDGGWDEPYYTGTFFPGDFYMGYTMYRHVFPTLALGRYKQAIERR

SEQ ID NO: 10 - protein, 680 aa, Streptomyces coelicolor
MTATTDGSTGASLRPLAASASDTDITIPAAAAGVPEAAARATRRATDFLLAKQDAEGWWKGDLETNVTMDAEDLLLRQFLGIQDEETTRAAALFIRGEQREDGTWATFYGGPGELSTTIEAYVALRLAGDSPEAPHMARAAEWIRSRGGIASARVFTRIWLALFGWWKWDDLPELPPELIYFPTWVPLNIYDFGCWARQTIVPLTIVSAKRPVRPAPFPLDELHTDPARPNPPRPLAPVASWDGAFQRIDKALHAYRKVAPRRLRRAAMNSAARWIIERQENDGCWGGIQPPAVYSVIALYLLGYDLEHPVMRAGLESLDRFAVWREDGARMIEACQSPVWDTCLATIALADAGVPEDHPQLVKASDWMLGEQIVRPGDWSVKRPGLPPGGWAAEFHNDNYPDIDDTAEVVLALRRVRHHDPERVEKAIGRGVRWNLGMQSKNGAWGAFDVDNTSAFPNRLPFCDFGEVIDPPSADVTAHVVEMLAVEGLAHDPRTRRGIQWLLDAQETDGSWFGRWGVNYVYGTGSVIPALTAAGLPTSHPAIRRAVRWLESVQNEDGGWGEDLRSYRYVREWSGRGASTASQTGWALMALLAAGERDSKAVERGVAWLAATQREDGSWDEPYFTGTGFPWDFSINYNLYRQVFPLTALGRYVHGEPFAKKPRAADAPAEAAPAEVKGS

SEQ ID NO: 11 - DNA, 1896 bp, Alicyclobacillus acidocaldarius
  source 1..1896: mol_type = unassigned DNA
atggcggaacagctggtggaagcgccggcgtatgcgcgcaccctggatcgcgcggtggaatatctgctgagctgccagaaagatgaaggctattggtggggcccgctgctgagcaacgtgaccatggaagcggaatatgtgctgctgtgccatattctggatcgcgtggatcgcgatcgcatggaaaaaattcgccgctatctgctgcatgaacagcgcgaagatggcacctgggcgctgtatccgggcggcccgccggatctggataccaccattgaagcgtatgtggcgctgaaatatattggcatgagccgcgatgaagaaccgatgcagaaagcgctgcgctttattcagagccagggcggcattgaaagcagccgcgtgtttacccgcatgtggctggcgctggtgggcgaatatccgtgggaaaaagtgccgatggtgccgccggaaattatgtttctgggcaaacgcatgccgctgaacatttatgaatttggcagctgggcgcgcgcgaccgtggtggcgctgagcattgtgatgagccgccagccggtgtttccgctgccggaacgcgcgcgcgtgccggaactgtatgaaaccgatgtgccgccgcgccgccgcggcgcgaaaggcggcggcggctggatttttgatgcgctggatcgcgcgctgcatggctatcagaaactgagcgtgcatccgtttcgccgcgcggcggaaattcgcgcgctggattggctgctggaacgccaggcgggcgatggcagctggggcggcattcagccgccgtggttttatgcgctgattgcgctgaaaattctggatatgacccagcatccggcgtttattaaaggctgggaaggcctggaactgtatggcgtggaactggattatggcggctggatgtttcaggcgagcattagcccggtgtgggataccggcctggcggtgctggcgctgcgcgcggcgggcctgccggcggatcatgatcgcctggtgaaagcgggcgaatggctgctggatcgccagattaccgtgccgggcgattgggcggtgaaacgcccgaacctgaaaccgggcggctttgcgtttcagtttgataacgtgtattatccggatgtggatgataccgcggtggtggtgtgggcgctgaacaccctgcgcctgccggatgaacgccgccgccgcgatgcgatgaccaaaggctttcgctggattgtgggcatgcagagcagcaacggcggctggggcgcgtatgatgtggataacaccagcgatctgccgaaccatattccgttttgcgattttggcgaagtgaccgatccgccgagcgaagatgtgaccgcgcatgtgctggaatgctttggcagctttggctatgatgatgcgtggaaagtgattcgccgcgcggtggaatatctgaaacgcgaacagaaaccggatggcagctggtttggccgctggggcgtgaactatctgtatggcaccggcgcggtggtgagcgcgctgaaagcggtgggcattgatacccgcgaaccgtatattcagaaagcgctggattgggtggaacagcatcagaacccggatggcggctggggcgaagattgccgcagctatgaagatccggcgtatgcgggcaaaggcgcgagcaccccgagccagaccgcgtgggcgctgatggcgctgattgcgggcggccgcgcggaaagcgaagcggcgcgccgcggcgtgcagtatctggtggaaacccagcgcccggatggcggctgggatgaaccgtattataccggcaccgggttcccgggcgatttttatctgggctataccatgtatcgccatgtgtttccgaccctggcgctgggccgctataaacaggcgattgaacgccgctaa